European Patent Application EP 4 729 941 A1, published April 22, 2026. Title: ONE-STEP PRECIPITATION AND COLOR DEVELOPMENT DETECTION METHOD OF nitrocellulose (NC) MEMBRANE FOR MICRO/NANO PLASTICS. Applicant: Wuhan Textile University. Application EP. The sequence listing filed with the application follows.

SEQUENCE LISTING (2 sequences)

SEQ ID NO: 1 - protein, 138 aa, synthetic construct
  source 1..138: note = the heavy chain variable region of the antibody
MEWSWIFLFLLSGTAGVHSEVQLQQSGPELVKPGASVKMSCKASGYTFTSYVMHWVKQKPGQGLEWIGYINPYNDGTKYNEKFKGKATLTSDKSSSTAYMELSSLTSEDSAVYYCASSYYYGSSYGYWGQGTTLTVSS

SEQ ID NO: 2 - protein, 127 aa, synthetic construct
  source 1..127: note = the light chain variable region of the antibody
MESQIQVFVFVFLWLSGVDGDIVMTQSHKFMSTSVGDRVSITCKASQDVSTAVAWYQQKPGQSPKLLIYSASYRYTGVPDRFTGSGSGTDFTFTISSVQAEDLAVYYCQQHYSTPLTFGAGTKLELK